European Patent Application EP 4 317 427 A1, published February 7, 2024. Title: MODIFIED LEVANSUCRASE FOR THE OPTIMIZED PRODUCTION OF FRUCTOOLIGOSACCHARIDES. Applicant: CENTRO DE INGENIERIA GENETICA Y BIOTECNOLOGIA. The sequence listing filed with the application follows.

SEQUENCE LISTING (34 sequences)

SEQ ID NO: 1 - DNA, 25 bp, Artificial Sequence
  Description of the Artificial Sequence: Oligonucleotide used as primer in the PCR
ggatcgtttcccatggcgcatgtac

SEQ ID NO: 2 - DNA, 33 bp, Artificial Sequence
  Description of the Artificial Sequence: Oligonucleotide used as primer in the mutagenesis of the lsdA gene
gatgcgggcatgcacgtgnnngtcgtcgaaacc

SEQ ID NO: 3 - DNA, 33 bp, Artificial Sequence
  Description of the Artificial Sequence: Oligonucleotide used as primer in the mutagenesis of the lsdA gene
gatgcgggcatgcacgctnnngtcgtcgaaacc

SEQ ID NO: 4 - DNA, 24 bp, Artificial Sequence
  Description of the Artificial Sequence: Oligonucleotide used as primer in the PCR
ctggggcggatccacgccgacttc

SEQ ID NO: 5 - DNA, 33 bp, Artificial Sequence
  Description of the Artificial Sequence: Oligonucleotide used as primer in the mutagenesis of the lsdA gene
gcgcagaacgaaaacttcaatttccgcgatccg

SEQ ID NO: 6 - DNA, 33 bp, Artificial Sequence
  Description of the Artificial Sequence: Oligonucleotide used as primer in the mutagenesis of the lsdA gene
cggatcgcggaaattgaagaattcgttctgcgc

SEQ ID NO: 7 - DNA, 33 bp, Artificial Sequence
  Description of the Artificial Sequence: Oligonucleotide used as primer in the mutagenesis of the lsdA gene
gcgcagaacgaatacttcaatttccgcgatccg

SEQ ID NO: 8 - DNA, 33 bp, Artificial Sequence
  Description of the Artificial Sequence: Oligonucleotide used as primer in the mutagenesis of the lsdA gene
cggatcgcggaaattgaagtattcgttctgcgc

SEQ ID NO: 9 - DNA, 33 bp, Artificial Sequence
  Description of the Artificial Sequence: Oligonucleotide used as primer in the mutagenesis of the lsdA gene
gcgcagaacgaatggttcaatttccgcgatccg

SEQ ID NO: 10 - DNA, 33 bp, Artificial Sequence
  Description of the Artificial Sequence: Oligonucleotide used as primer in the mutagenesis of the lsdA gene
cggatcgcggaaattgaaccattcgttctgcgc

SEQ ID NO: 11 - DNA, 24 bp, Artificial Sequence
  Description of the Artificial Sequence: Oligonucleotide used as primer in the PCR
ggcgccagggtacccccgcgacgg

SEQ ID NO: 12 - DNA, 27 bp, Artificial Sequence
  Description of the Artificial Sequence: Oligonucleotide used as primer in the mutagenesis of the lsdA gene
cgcagaacgaattcttcnnnttccgcg

SEQ ID NO: 13 - DNA, 33 bp, Artificial Sequence
  Description of the Artificial Sequence: Oligonucleotide used as primer in the mutagenesis of the lsdA gene
ggcaataccgcgggccagcatggcgtcgccaac

SEQ ID NO: 14 - DNA, 33 bp, Artificial Sequence
  Description of the Artificial Sequence: Oligonucleotide used as primer in the mutagenesis of the lsdA gene
gttggcgacgccatgctggcccgcggtattgcc

SEQ ID NO: 15 - DNA, 33 bp, Artificial Sequence
  Description of the Artificial Sequence: Oligonucleotide used as primer in the mutagenesis of the lsdA gene
ggcaataccgcgggccagaagggcgtcgccaac

SEQ ID NO: 16 - DNA, 33 bp, Artificial Sequence
  Description of the Artificial Sequence: Oligonucleotide used as primer in the mutagenesis of the lsdA gene
gttggcgacgcccttctggcccgcggtattgcc

SEQ ID NO: 17 - DNA, 33 bp, Artificial Sequence
  Description of the Artificial Sequence: Oligonucleotide used as primer in the mutagenesis of the lsdA gene
ggcaataccgcgggccagtcgggcgtcgccaac

SEQ ID NO: 18 - DNA, 33 bp, Artificial Sequence
  Description of the Artificial Sequence: Oligonucleotide used as primer in the mutagenesis of the lsdA gene
gttggcgacgcccgactggcccgcggtattgcc

SEQ ID NO: 19 - DNA, 33 bp, Artificial Sequence
  Description of the Artificial Sequence: Oligonucleotide used as primer in the mutagenesis of the lsdA gene
ggcaataccgcgggccaggccggcgtcgccaac

SEQ ID NO: 20 - DNA, 33 bp, Artificial Sequence
  Description of the Artificial Sequence: Oligonucleotide used as primer in the mutagenesis of the lsdA gene
gttggcgacgccggcctggcccgcggtattgcc

SEQ ID NO: 21 - DNA, 27 bp, Artificial Sequence
  Description of the Artificial Sequence: Oligonucleotide used as primer en la mutagenesis del gen lsdA
cgcagaacgaattcttccacttccgcg

SEQ ID NO: 22 - DNA, 27 bp, Artificial Sequence
  Description of the Artificial Sequence: Oligonucleotide used as primer in the mutagenesis of the lsdA gene
cgcagaacgaattcttccgcttccgcg

SEQ ID NO: 23 - DNA, 27 bp, Artificial Sequence
  Description of the Artificial Sequence: Oligonucleotide used as primer in the mutagenesis of the lsdA gene
cgcagaacgaattcttcaagttccgcg

SEQ ID NO: 24 - DNA, 27 bp, Artificial Sequence
  Description of the Artificial Sequence: Oligonucleotide used as primer in the PCR
agtgcgctatcgatagggaatttcagc

SEQ ID NO: 25 - DNA, 27 bp, Artificial Sequence
  Description of the Artificial Sequence: Oligonucleotide used as primer in the PCR
ttactggtctagaaattggcgaacctg

SEQ ID NO: 26 - protein, 554 aa, Artificial Sequence
  Description of the Artificial Sequence: Modified Levansucrase H142E
QGNFSRQEAARMAHRPGVMPRGGPLFPGRSLAGVPGFPLPSIHTQQAYDPQSDFTARWTRADALQIKAHSDATVAAGQNSLPAQLTMPNIPADFPVINPDVWVWDTWTLIDKHADQFSYNGWEVIFCLTADPNAGYGFDDREVHARIGFFYRRAGIPASRRPVNGGWTYGGHLFPDGASAQVYAGQTYTNQAEWSGSSRLMQIHGNTVSVFYTDVAFNRDANANNITPPQAIITQTLGRIHADFNHVWFTGFTAHTPLLQPDGVLYQNGAQNEFFNFRDPFTFEDPKHPGVNYMVFEGNTAGQRGVANCTEADLGFRPNDPNAETLQEVLDSGAYYQKANIGLAIATDSTLSKWKFLSPLISANCVNDQTERPQVYLHNGKYYIFTISHRTTFAAGVDGPDGVYGFVGDGIRSDFQPMNYGSGLTMGNPTDLNTAAGTDFDPSPDQNPRAFQSYSHYVMPGGLVESFIDTVENRRGGTLAPTVRVRIAQNASAVDLRYGNGGLGGYGDIPANRADVNIAGFIQDLFGQPTSGLAAQASTNNAQVLAQVRQFLNQ

SEQ ID NO: 27 - protein, 554 aa, Artificial Sequence
  Description of the Artificial Sequence: Modified Levansucrase R141K-H142S
QGNFSRQEAARMAHRPGVMPRGGPLFPGRSLAGVPGFPLPSIHTQQAYDPQSDFTARWTRADALQIKAHSDATVAAGQNSLPAQLTMPNIPADFPVINPDVWVWDTWTLIDKHADQFSYNGWEVIFCLTADPNAGYGFDDKSVHARIGFFYRRAGIPASRRPVNGGWTYGGHLFPDGASAQVYAGQTYTNQAEWSGSSRLMQIHGNTVSVFYTDVAFNRDANANNITPPQAIITQTLGRIHADFNHVWFTGFTAHTPLLQPDGVLYQNGAQNEFFNFRDPFTFEDPKHPGVNYMVFEGNTAGQRGVANCTEADLGFRPNDPNAETLQEVLDSGAYYQKANIGLAIATDSTLSKWKFLSPLISANCVNDQTERPQVYLHNGKYYIFTISHRTTFAAGVDGPDGVYGFVGDGIRSDFQPMNYGSGLTMGNPTDLNTAAGTDFDPSPDQNPRAFQSYSHYVMPGGLVESFIDTVENRRGGTLAPTVRVRIAQNASAVDLRYGNGGLGGYGDIPANRADVNIAGFIQDLFGQPTSGLAAQASTNNAQVLAQVRQFLNQ

SEQ ID NO: 28 - protein, 554 aa, Artificial Sequence
  Description of the Artificial Sequence: Modified Levansucrase F274A
QGNFSRQEAARMAHRPGVMPRGGPLFPGRSLAGVPGFPLPSIHTQQAYDPQSDFTARWTRADALQIKAHSDATVAAGQNSLPAQLTMPNIPADFPVINPDVWVWDTWTLIDKHADQFSYNGWEVIFCLTADPNAGYGFDDRHVHARIGFFYRRAGIPASRRPVNGGWTYGGHLFPDGASAQVYAGQTYTNQAEWSGSSRLMQIHGNTVSVFYTDVAFNRDANANNITPPQAIITQTLGRIHADFNHVWFTGFTAHTPLLQPDGVLYQNGAQNEAFNFRDPFTFEDPKHPGVNYMVFEGNTAGQRGVANCTEADLGFRPNDPNAETLQEVLDSGAYYQKANIGLAIATDSTLSKWKFLSPLISANCVNDQTERPQVYLHNGKYYIFTISHRTTFAAGVDGPDGVYGFVGDGIRSDFQPMNYGSGLTMGNPTDLNTAAGTDFDPSPDQNPRAFQSYSHYVMPGGLVESFIDTVENRRGGTLAPTVRVRIAQNASAVDLRYGNGGLGGYGDIPANRADVNIAGFIQDLFGQPTSGLAAQASTNNAQVLAQVRQFLNQ

SEQ ID NO: 29 - protein, 554 aa, Artificial Sequence
  Description of the Artificial Sequence: Modified Levansucrase N276H
QGNFSRQEAARMAHRPGVMPRGGPLFPGRSLAGVPGFPLPSIHTQQAYDPQSDFTARWTRADALQIKAHSDATVAAGQNSLPAQLTMPNIPADFPVINPDVWVWDTWTLIDKHADQFSYNGWEVIFCLTADPNAGYGFDDRHVHARIGFFYRRAGIPASRRPVNGGWTYGGHLFPDGASAQVYAGQTYTNQAEWSGSSRLMQIHGNTVSVFYTDVAFNRDANANNITPPQAIITQTLGRIHADFNHVWFTGFTAHTPLLQPDGVLYQNGAQNEFFHFRDPFTFEDPKHPGVNYMVFEGNTAGQRGVANCTEADLGFRPNDPNAETLQEVLDSGAYYQKANIGLAIATDSTLSKWKFLSPLISANCVNDQTERPQVYLHNGKYYIFTISHRTTFAAGVDGPDGVYGFVGDGIRSDFQPMNYGSGLTMGNPTDLNTAAGTDFDPSPDQNPRAFQSYSHYVMPGGLVESFIDTVENRRGGTLAPTVRVRIAQNASAVDLRYGNGGLGGYGDIPANRADVNIAGFIQDLFGQPTSGLAAQASTNNAQVLAQVRQFLNQ

SEQ ID NO: 30 - protein, 554 aa, Artificial Sequence
  Description of the Artificial Sequence: Modified Levansucrase N276R
QGNFSRQEAARMAHRPGVMPRGGPLFPGRSLAGVPGFPLPSIHTQQAYDPQSDFTARWTRADALQIKAHSDATVAAGQNSLPAQLTMPNIPADFPVINPDVWVWDTWTLIDKHADQFSYNGWEVIFCLTADPNAGYGFDDRHVHARIGFFYRRAGIPASRRPVNGGWTYGGHLFPDGASAQVYAGQTYTNQAEWSGSSRLMQIHGNTVSVFYTDVAFNRDANANNITPPQAIITQTLGRIHADFNHVWFTGFTAHTPLLQPDGVLYQNGAQNEFFRFRDPFTFEDPKHPGVNYMVFEGNTAGQRGVANCTEADLGFRPNDPNAETLQEVLDSGAYYQKANIGLAIATDSTLSKWKFLSPLISANCVNDQTERPQVYLHNGKYYIFTISHRTTFAAGVDGPDGVYGFVGDGIRSDFQPMNYGSGLTMGNPTDLNTAAGTDFDPSPDQNPRAFQSYSHYVMPGGLVESFIDTVENRRGGTLAPTVRVRIAQNASAVDLRYGNGGLGGYGDIPANRADVNIAGFIQDLFGQPTSGLAAQASTNNAQVLAQVRQFLNQ

SEQ ID NO: 31 - protein, 554 aa, Artificial Sequence
  Description of the Artificial Sequence: Modified Levansucrase R304K
QGNFSRQEAARMAHRPGVMPRGGPLFPGRSLAGVPGFPLPSIHTQQAYDPQSDFTARWTRADALQIKAHSDATVAAGQNSLPAQLTMPNIPADFPVINPDVWVWDTWTLIDKHADQFSYNGWEVIFCLTADPNAGYGFDDRHVHARIGFFYRRAGIPASRRPVNGGWTYGGHLFPDGASAQVYAGQTYTNQAEWSGSSRLMQIHGNTVSVFYTDVAFNRDANANNITPPQAIITQTLGRIHADFNHVWFTGFTAHTPLLQPDGVLYQNGAQNEFFNFRDPFTFEDPKHPGVNYMVFEGNTAGQKGVANCTEADLGFRPNDPNAETLQEVLDSGAYYQKANIGLAIATDSTLSKWKFLSPLISANCVNDQTERPQVYLHNGKYYIFTISHRTTFAAGVDGPDGVYGFVGDGIRSDFQPMNYGSGLTMGNPTDLNTAAGTDFDPSPDQNPRAFQSYSHYVMPGGLVESFIDTVENRRGGTLAPTVRVRIAQNASAVDLRYGNGGLGGYGDIPANRADVNIAGFIQDLFGQPTSGLAAQASTNNAQVLAQVRQFLNQ

SEQ ID NO: 32 - protein, 554 aa, Artificial Sequence
  Description of the Artificial Sequence: Modified Levansucrase N276H-R304K
QGNFSRQEAARMAHRPGVMPRGGPLFPGRSLAGVPGFPLPSIHTQQAYDPQSDFTARWTRADALQIKAHSDATVAAGQNSLPAQLTMPNIPADFPVINPDVWVWDTWTLIDKHADQFSYNGWEVIFCLTADPNAGYGFDDRHVHARIGFFYRRAGIPASRRPVNGGWTYGGHLFPDGASAQVYAGQTYTNQAEWSGSSRLMQIHGNTVSVFYTDVAFNRDANANNITPPQAIITQTLGRIHADFNHVWFTGFTAHTPLLQPDGVLYQNGAQNEFFHFRDPFTFEDPKHPGVNYMVFEGNTAGQKGVANCTEADLGFRPNDPNAETLQEVLDSGAYYQKANIGLAIATDSTLSKWKFLSPLISANCVNDQTERPQVYLHNGKYYIFTISHRTTFAAGVDGPDGVYGFVGDGIRSDFQPMNYGSGLTMGNPTDLNTAAGTDFDPSPDQNPRAFQSYSHYVMPGGLVESFIDTVENRRGGTLAPTVRVRIAQNASAVDLRYGNGGLGGYGDIPANRADVNIAGFIQDLFGQPTSGLAAQASTNNAQVLAQVRQFLNQ

SEQ ID NO: 33 - protein, 554 aa, Artificial Sequence
  Description of the Artificial Sequence: Modified Levansucrase N276R-R304K
QGNFSRQEAARMAHRPGVMPRGGPLFPGRSLAGVPGFPLPSIHTQQAYDPQSDFTARWTRADALQIKAHSDATVAAGQNSLPAQLTMPNIPADFPVINPDVWVWDTWTLIDKHADQFSYNGWEVIFCLTADPNAGYGFDDRHVHARIGFFYRRAGIPASRRPVNGGWTYGGHLFPDGASAQVYAGQTYTNQAEWSGSSRLMQIHGNTVSVFYTDVAFNRDANANNITPPQAIITQTLGRIHADFNHVWFTGFTAHTPLLQPDGVLYQNGAQNEFFRFRDPFTFEDPKHPGVNYMVFEGNTAGQKGVANCTEADLGFRPNDPNAETLQEVLDSGAYYQKANIGLAIATDSTLSKWKFLSPLISANCVNDQTERPQVYLHNGKYYIFTISHRTTFAAGVDGPDGVYGFVGDGIRSDFQPMNYGSGLTMGNPTDLNTAAGTDFDPSPDQNPRAFQSYSHYVMPGGLVESFIDTVENRRGGTLAPTVRVRIAQNASAVDLRYGNGGLGGYGDIPANRADVNIAGFIQDLFGQPTSGLAAQASTNNAQVLAQVRQFLNQ

SEQ ID NO: 34 - protein, 554 aa, Artificial Sequence
  Description of the Artificial Sequence: Modified Levansucrase N276K-R304K
QGNFSRQEAARMAHRPGVMPRGGPLFPGRSLAGVPGFPLPSIHTQQAYDPQSDFTARWTRADALQIKAHSDATVAAGQNSLPAQLTMPNIPADFPVINPDVWVWDTWTLIDKHADQFSYNGWEVIFCLTADPNAGYGFDDRHVHARIGFFYRRAGIPASRRPVNGGWTYGGHLFPDGASAQVYAGQTYTNQAEWSGSSRLMQIHGNTVSVFYTDVAFNRDANANNITPPQAIITQTLGRIHADFNHVWFTGFTAHTPLLQPDGVLYQNGAQNEFFKFRDPFTFEDPKHPGVNYMVFEGNTAGQKGVANCTEADLGFRPNDPNAETLQEVLDSGAYYQKANIGLAIATDSTLSKWKFLSPLISANCVNDQTERPQVYLHNGKYYIFTISHRTTFAAGVDGPDGVYGFVGDGIRSDFQPMNYGSGLTMGNPTDLNTAAGTDFDPSPDQNPRAFQSYSHYVMPGGLVESFIDTVENRRGGTLAPTVRVRIAQNASAVDLRYGNGGLGGYGDIPANRADVNIAGFIQDLFGQPTSGLAAQASTNNAQVLAQVRQFLNQ